European Patent Application EP 4 613 874 A1, published September 10, 2025. Title: Sequencing Adapter, Sequencing Adapter Complex, Method for Multiple Amplifications of Target Nucleic Acid Sequence, and Method for Nanopore Sequencing. Applicant: BGI SHENZHEN. Application CN. The sequence listing filed with the application follows.

SEQUENCE LISTING (7 sequences)

SEQ ID NO: 1 - DNA, 473 bp, synthetic construct
  source 1..473: mol_type = other DNA
gaattcgccatcagattgtgtttgttagtcgctttttttttttggaattttttttttggaattttttttttgcgctaacaacctcctgccgttttgcccgtgcatatcggtcacgaacaaatctgattactaaacacagtagcctggatttgttctatcagtaatcgaccttattcctaattaaatagagcaaatccccttattgggggtaagacatgaagatgccagaaaaacatgacctgttggccgccattctcgcggcaaaggaacaaggcatcggggcaatccttgcgtttgcaatggcgtaccttcgcggcagatataatggcggtgcgtttacaaaaacagtaatcgacgcaacgatgtgcgccattatcgcctagttcattcgtgaccttctcgacttcgccggactaagtagcaatctcgcttatataacgagcgtgtttatcggctacatcggtactgactcg

SEQ ID NO: 2 - DNA, 93 bp, synthetic construct
  source 1..93: mol_type = other DNA
  misc_feature 1: note = Phosphorylation modification
tgcaatacgtaactgaacgaagtacattttttttccttggctcacagaacgacatggctttttttttgtacttcgttcagttacgtattgcat

SEQ ID NO: 3 - DNA, 96 bp, synthetic construct
  source 1..96: mol_type = other DNA
  misc_feature 1..30: note = N = iSpC3
  misc_feature 41..44: note = Y = iSp18
nnnnnnnnnnnnnnnnnnnnnnnnnnnnnnttttttttttyyyyggttgtttctgttggtgctgatattgctgccatgtcgttctgtgagccaagg

SEQ ID NO: 4 - DNA, 43 bp, synthetic construct
  source 1..43: mol_type = other DNA
  misc_feature 1..4: note = LNA modification
aatatcagcaccaacagaaacaacctttgaggcgagcggtcaa

SEQ ID NO: 5 - protein, 442 aa, synthetic construct
GSHGTFDDLTEGQKNAFNIVMKAIKEKKHHVTINGPAGTGKTTLTKFIIEALISTGETGIILAAPTHAAKKILSKLSGKEASTIHSILKINPVTYECNVLFEQKEVPDLAKARVLICDEVSMYDRKLFKILLSTIPPWATIIGIGDNKQIRPVDPGENTAYISPFFTHKDFYQCELTEVKRSNAPIIDVATDVRNGLWIYDKVVDGHGVRGFTGDTALRDFMVNYFSIVKSLDDLFENRVMAFTNKSVDKLNSIIRKKIFETDKDFIVGEIIVMQEPLFKTYKIDGKPVSEIIFNNGQLVRIIEAEYTSTFVKARGVPGEYLIRHWDLTVETYGDDEYYREKIKIISSDEELYKFNLFLGKTCETYKNWNKGGKAPWSDFWDAKSQFSKVKALPASTFHKAQGMSVDRAFIYTPCIHYADVELAQQLLYVGVTRGRYDVFYV

SEQ ID NO: 6 - DNA, 24 bp, synthetic construct
  source 1..24: mol_type = other DNA
  misc_feature 1..4: note = LNA modification
ccttggctcacagaacgacatggc

SEQ ID NO: 7 - DNA, 16 bp, synthetic construct
  source 1..16: mol_type = other DNA
  misc_feature 1..4: note = Y=iSp18
  misc_feature 1: note = Cholesterol modification
yyyyttgaccgctcgc